European Patent Specification EP 4 063 497 B1, published April 24, 2024. Title: IMP-TYPE CARBAPENEMASE-RESISTANT HYBRIDOMA CELL LINE, AND MONOCLONAL ANTIBODY (mAb) AND USE THEREOF. Applicant: TIANJIN ERA BIOLOGY TECHNOLOGY CO., LTD. BEIJING GOLD MOUNTAINRIVER TECH DEVELOPMENT CO., LTD. The sequence listing filed with the application follows.

SEQUENCE LISTING (24 sequences)

SEQ ID NO: 1 - protein, 16 aa, Artificial Sequence
  The sequence is synthetized.
RSSQSLLDSGGKTYLN

SEQ ID NO: 2 - protein, 6 aa, Artificial Sequence
  The sequence is synthetized.
YLVSKL

SEQ ID NO: 3 - protein, 10 aa, Artificial Sequence
  The sequence is synthetized.
FQYTHFPQCT

SEQ ID NO: 4 - protein, 13 aa, Artificial Sequence
  The sequence is synthetized.
AASGFTFSDYYMY

SEQ ID NO: 5 - protein, 19 aa, Artificial Sequence
  The sequence is synthetized.
VAIISDGGSYTYYPDSVKG

SEQ ID NO: 6 - protein, 7 aa, Artificial Sequence
  The sequence is synthetized.
VRGSFDV

SEQ ID NO: 7 - protein, 115 aa, Artificial Sequence
  The sequence is synthetized.
DIVMTQSPLTLSVTLGQPASISCRSSQSLLDSGGKTYLNWFLQRPGQSPKRLIYLVSKLDSGVPDRFTGSGSGTDFTLRISRVEAEDLGIYYCFQYTHFPQCTFGGGTTLEIKRA

SEQ ID NO: 8 - DNA, 345 bp, Artificial Sequence
  The sequence is synthetized.
gacattgtcatgacccagtctccactcactttgtcggttacccttggacaaccagcctccatctcttgcaggtcaagtcagagcctcttagatagtggtggaaagacatatttgaattggtttttacagaggccaggccagtctccaaagcgcctaatctatctggtgtctaaactggactctggagtccctgacaggttcactggcagtggatcagggacagatttcacactgagaatcagcagagtggaggctgaggatttgggaatttattattgcttccaatatacacattttcctcagtgtacgttcggaggggggaccacgctggaaatcaaacgggct

SEQ ID NO: 9 - protein, 113 aa, Artificial Sequence
  The sequence is synthetized.
VQLVVSGGGLVNPDGSLKLSCAASGFTFSDYYMYWVRQTPEKRLEWVAIISDGGSYTYYPDSVKGRFTISRDNAKNNLYLQMSGLRSEDTAMYYCVRGSFDVWGAGTTVTVSA

SEQ ID NO: 10 - DNA, 341 bp, Artificial Sequence
  The sequence is synthetized.
gtgcagttggtggtgtctgggggaggcttagtgaaccctgacgggtccctgaaactctcctgtgcagcctctggattcactttcagtgactattacatgtattgggttcgccagactccggaaaagaggctggagtgggtcgctataattagtgatggtggttcttacacctactatccagacagtgtgaaggggcgattcaccatctccagagacaatgccaagaataatttgtacctgcaaatgagcggtctgaggtctgaggacacggccatgtattattgtgtaagagggtcattcgatgtctggggcgcagggaccacggtcaccgtctctgcagc

SEQ ID NO: 11 - protein, 17 aa, Artificial Sequence
  The sequence is synthetized.
KSSQSLLNSGHQKNYLA

SEQ ID NO: 12 - protein, 7 aa, Artificial Sequence
  The sequence is synthetized.
YGASTRK

SEQ ID NO: 13 - protein, 9 aa, Artificial Sequence
  The sequence is synthetized.
QNDHRYPLT

SEQ ID NO: 14 - protein, 13 aa, Artificial Sequence
  The sequence is synthetized.
KASGYTFTDYNMD

SEQ ID NO: 15 - protein, 19 aa, Artificial Sequence
  The sequence is synthetized.
IGDINPNYDSTRYNQKFKG

SEQ ID NO: 16 - protein, 10 aa, Artificial Sequence
  The sequence is synthetized.
ARDGRYAMDY

SEQ ID NO: 17 - protein, 115 aa, Artificial Sequence
  The sequence is synthetized.
DIVMTQSPSSLSVSAGEKVTLTCKSSQSLLNSGHQKNYLAWYQQKPGQPPKLLIYGASTRKSGIPDRFTGSGSGTDFTLTISSVQAEDLAVYYCQNDHRYPLTFGAGTKLELKRA

SEQ ID NO: 18 - DNA, 347 bp, Artificial Sequence
  The sequence is synthetized.
gacattgtcatgacacagtctccatcctccctgagtgtgtcagcaggagagaaggtcactttgacctgcaagtccagtcagagtctgttaaacagtggacatcaaaagaactacttggcctggtaccagcagaaaccagggcagcctcctaaactgttgatctacggggcatccactaggaaatctgggatccctgatcgcttcacaggcagtggatctggaaccgatttcactcttaccatcagcagtgtgcaggctgaagacctggcagtttattactgtcagaatgatcatcgttatcctctcacgttcggtgctgggaccaagctggagctgaaacgggctga

SEQ ID NO: 19 - protein, 116 aa, Artificial Sequence
  The sequence is synthetized.
VKLQQSGAELVKPGASVKISCKASGYTFTDYNMDWVKQSHGKSLEWIGDINPNYDSTRYNQKFKGKATLTVDKSSSTAYMELRSLTSEDTAVYYCARDGRYAMDYWGQGTSVTVSS

SEQ ID NO: 20 - DNA, 348 bp, Artificial Sequence
  The sequence is synthetized.
gtgaagcttcagcagtctggagctgagctggtgaagcctggggcttcagtgaagatatcctgcaaggcttctggctacacattcactgactacaacatggactgggtgaagcagagccatggaaagagccttgagtggattggagatattaatcctaactatgatagtactaggtacaaccagaagttcaagggaaaggccacattgactgtagacaagtcctccagcacagcctacatggagctccgcagcctgacatctgaggacactgcagtctattactgtgcaagagacggccgctatgctatggactactggggtcaaggaacctcagtcaccgtctcttca

SEQ ID NO: 21 - DNA, 23 bp, Artificial Sequence
  Upstream primer for a heavy chain framework region
saggtgmagctkcassartcwgg

SEQ ID NO: 22 - DNA, 32 bp, Artificial Sequence
  Downstream primer for a heavy chain variable region
tggggstgtygttttggctgmrgagacrgtga

SEQ ID NO: 23 - DNA, 26 bp, Artificial Sequence
  Upstream primer for a light chain leader peptide
atggattttcaagtgcagattttcag

SEQ ID NO: 24 - DNA, 30 bp, Artificial Sequence
  Downstream primer for a light chain variable region
ggatacagttggtgcagcatcagcccgttt